European Patent Specification EP 3 864 028 B1, published March 25, 2026. Title: OLIGONUCLEOTIDE-BASED TUNING OF PORE-FORMING PEPTIDES FOR INCREASING PORE SIZE, MEMBRANE AFFINITY, STABILITY, AND ANTIMICROBIAL ACTIVITY. Applicant: Adolphe Merkle Institute, University of Fribourg. The sequence listing filed with the application follows.

SEQUENCE LISTING (197 sequences)

SEQ ID NO: 1 - protein, 36 aa, Artificial Sequence
  Synthetic peptide
SIGSALKKALPVAKKIGKIALPIAKAALPVAAGLVG

SEQ ID NO: 2 - DNA, 55 bp, Artificial Sequence
  Synthetic oligonucleotide
tttttcagcaatttaagatccacccacgtttttgtcacttccgcgcaccagtttt

SEQ ID NO: 3 - DNA, 33 bp, Artificial Sequence
  Synthetic oligonucleotide
ttttacgtgggtggatcttaaattgctgatttt

SEQ ID NO: 4 - DNA, 22 bp, Artificial Sequence
  Synthetic oligonucleotide
ctggtgcgcggaagtgactttt

SEQ ID NO: 5 - DNA, 28 bp, Artificial Sequence
  Synthetic oligonucleotide
gcagaagccgcctgcaacagtgagatct

SEQ ID NO: 6 - DNA, 28 bp, Artificial Sequence
  Synthetic oligonucleotide
taagaatatagtgagagcaaaagaagat

SEQ ID NO: 7 - DNA, 28 bp, Artificial Sequence
  Synthetic oligonucleotide
ttatagtgggtgcctaatgagtgagctt

SEQ ID NO: 8 - DNA, 36 bp, Artificial Sequence
  Synthetic oligonucleotide
ttaaatcccttataaatcggttccgaaatcggcatt

SEQ ID NO: 9 - DNA, 36 bp, Artificial Sequence
  Synthetic oligonucleotide
ttaccagtaataaaagggattcaccagtcacacgtt

SEQ ID NO: 10 - DNA, 42 bp, Artificial Sequence
  Synthetic oligonucleotide
ggaagcctccacactcgctatgcactccaggaacgccatcaa

SEQ ID NO: 11 - DNA, 35 bp, Artificial Sequence
  Synthetic oligonucleotide
atttatccaatccattatccggtattctaaaataa

SEQ ID NO: 12 - DNA, 42 bp, Artificial Sequence
  Synthetic oligonucleotide
ttcattgaatccccttaaacaattgcataagcatagggcgat

SEQ ID NO: 13 - DNA, 28 bp, Artificial Sequence
  Synthetic oligonucleotide
ctcaaactcatcgagaacaagttaaacc

SEQ ID NO: 14 - DNA, 28 bp, Artificial Sequence
  Synthetic oligonucleotide
gcttcaacttcaaatccaagaacgggta

SEQ ID NO: 15 - DNA, 42 bp, Artificial Sequence
  Synthetic oligonucleotide
tatcgcgttatcatatgcgtttcggctgtctttccgtaggaa

SEQ ID NO: 16 - DNA, 42 bp, Artificial Sequence
  Synthetic oligonucleotide
gtcagtttacgtggcacagacgaacaaacggcgtacctacat

SEQ ID NO: 17 - DNA, 32 bp, Artificial Sequence
  Synthetic oligonucleotide
ttttataatcagtgaggccaccgagataagag

SEQ ID NO: 18 - DNA, 42 bp, Artificial Sequence
  Synthetic oligonucleotide
aaaagaatagcccgccggaaagcaactgagagaatcgatgaa

SEQ ID NO: 19 - DNA, 28 bp, Artificial Sequence
  Synthetic oligonucleotide
caaaatatttttattttcatcttatcat

SEQ ID NO: 20 - DNA, 28 bp, Artificial Sequence
  Synthetic oligonucleotide
aatattttcaatcaatatctgcctttgc

SEQ ID NO: 21 - DNA, 28 bp, Artificial Sequence
  Synthetic oligonucleotide
ctcaacaaatttttagaaccctcatatt

SEQ ID NO: 22 - DNA, 42 bp, Artificial Sequence
  Synthetic oligonucleotide
acaataaattagttaatcttaccaacgctgtaaatatatttt

SEQ ID NO: 23 - DNA, 35 bp, Artificial Sequence
  Synthetic oligonucleotide
gttgagtgttgttctttccggcggtgcgcctgaga

SEQ ID NO: 24 - DNA, 28 bp, Artificial Sequence
  Synthetic oligonucleotide
tagagctgcgcgtactatggtcgttaga

SEQ ID NO: 25 - DNA, 28 bp, Artificial Sequence
  Synthetic oligonucleotide
aataaccaaggcaaagaattaggagcgg

SEQ ID NO: 26 - DNA, 42 bp, Artificial Sequence
  Synthetic oligonucleotide
agccctaaaatctaaagcatctatcatttttaaattaatgcc

SEQ ID NO: 27 - DNA, 36 bp, Artificial Sequence
  Synthetic oligonucleotide
ttttagagccgtcaatagactaacaactaatagatt

SEQ ID NO: 28 - DNA, 49 bp, Artificial Sequence
  Synthetic oligonucleotide
tgcgtaggcacgtaaaacagaaaaattctactaatagtagtaaattcat

SEQ ID NO: 29 - DNA, 42 bp, Artificial Sequence
  Synthetic oligonucleotide
aattatcttattaacaaacccttgaatggctattaaacccgt

SEQ ID NO: 30 - DNA, 28 bp, Artificial Sequence
  Synthetic oligonucleotide
ggttgataatcagagcaaacattgggaa

SEQ ID NO: 31 - DNA, 36 bp, Artificial Sequence
  Synthetic oligonucleotide
ttaacctaccatatcaaaataatggaagggttagtt

SEQ ID NO: 32 - DNA, 28 bp, Artificial Sequence
  Synthetic oligonucleotide
agatagggcgaaaatcctgtttgatggt

SEQ ID NO: 33 - DNA, 35 bp, Artificial Sequence
  Synthetic oligonucleotide
ccggcttctaatttccgacttgcgggaggaacgcg

SEQ ID NO: 34 - DNA, 28 bp, Artificial Sequence
  Synthetic oligonucleotide
tattaaaagagagttgcagcaagctgca

SEQ ID NO: 35 - DNA, 37 bp, Artificial Sequence
  Synthetic oligonucleotide
ttagtttgaccattgatgaaacaaacatacagtgccc

SEQ ID NO: 36 - DNA, 35 bp, Artificial Sequence
  Synthetic oligonucleotide
aactatataacgagagccttaaatcaagacaacat

SEQ ID NO: 37 - DNA, 36 bp, Artificial Sequence
  Synthetic oligonucleotide
tttcgccattcaggctgcccaggcaaagcgccattt

SEQ ID NO: 38 - DNA, 28 bp, Artificial Sequence
  Synthetic oligonucleotide
acgacgtgatccccgggtacccgctcaa

SEQ ID NO: 39 - DNA, 33 bp, Artificial Sequence
  Synthetic oligonucleotide
ggaaacgataccaagcgcggacagcctttcgag

SEQ ID NO: 40 - DNA, 42 bp, Artificial Sequence
  Synthetic oligonucleotide
gagagacaaacagccgaggcgttttagcatagatatttaaca

SEQ ID NO: 41 - DNA, 46 bp, Artificial Sequence
  Synthetic oligonucleotide
ttagtaacagtaccttttacatcggcaaatccaatcgcaagacatt

SEQ ID NO: 42 - DNA, 28 bp, Artificial Sequence
  Synthetic oligonucleotide
tagtaataccgttggaggccgattaaag

SEQ ID NO: 43 - DNA, 42 bp, Artificial Sequence
  Synthetic oligonucleotide
tcacaatcgaaagaagcgaacaattttctttgaattaccttt

SEQ ID NO: 44 - DNA, 35 bp, Artificial Sequence
  Synthetic oligonucleotide
aatcatgttcttactaattacttaagacgctgaga

SEQ ID NO: 45 - DNA, 22 bp, Artificial Sequence
  Synthetic oligonucleotide
acgaaggcaccaaccttaaacg

SEQ ID NO: 46 - DNA, 28 bp, Artificial Sequence
  Synthetic oligonucleotide
cgttctagctgagcggaacaaggaatca

SEQ ID NO: 47 - DNA, 36 bp, Artificial Sequence
  Synthetic oligonucleotide
ttaaagtaattctgtccaagtaccgacaaaaggttt

SEQ ID NO: 48 - DNA, 28 bp, Artificial Sequence
  Synthetic oligonucleotide
gtaagaaggcaaatcaacagtattcgac

SEQ ID NO: 49 - DNA, 28 bp, Artificial Sequence
  Synthetic oligonucleotide
gttttgacgtctttccagagcaggttgg

SEQ ID NO: 50 - DNA, 28 bp, Artificial Sequence
  Synthetic oligonucleotide
agatacataagcaataaagcctcagagc

SEQ ID NO: 51 - DNA, 35 bp, Artificial Sequence
  Synthetic oligonucleotide
acattctatatctttaggagcataatacatttgag

SEQ ID NO: 52 - DNA, 28 bp, Artificial Sequence
  Synthetic oligonucleotide
ttccaatactgcggaatcgtcaatgacc

SEQ ID NO: 53 - DNA, 42 bp, Artificial Sequence
  Synthetic oligonucleotide
aagccaagagctcggggttttcgcatcgtgtgagcgagtaac

SEQ ID NO: 54 - DNA, 39 bp, Artificial Sequence
  Synthetic oligonucleotide
tttgataagaggtcatttttgagtgaataaccgggtaat

SEQ ID NO: 55 - DNA, 28 bp, Artificial Sequence
  Synthetic oligonucleotide
aagtgtaactgcccgctttccccagcag

SEQ ID NO: 56 - DNA, 42 bp, Artificial Sequence
  Synthetic oligonucleotide
tcaaaaggaagcctgtacggtgtctggatttaatgcgtcgct

SEQ ID NO: 57 - DNA, 49 bp, Artificial Sequence
  Synthetic oligonucleotide
aacgccaaattcgttgggcgccagggtggtttttataacgtgctttcct

SEQ ID NO: 58 - DNA, 32 bp, Artificial Sequence
  Synthetic oligonucleotide
gtgaatttaaggctccaaaaggagcatttaac

SEQ ID NO: 59 - DNA, 28 bp, Artificial Sequence
  Synthetic oligonucleotide
aaaggtggcatctaaagaaatgattcgc

SEQ ID NO: 60 - DNA, 46 bp, Artificial Sequence
  Synthetic oligonucleotide
cttctgaattatttattttcaggtttaacgtcagatgaatatactt

SEQ ID NO: 61 - DNA, 28 bp, Artificial Sequence
  Synthetic oligonucleotide
gtacccctaaattgtaaacgttaatatt

SEQ ID NO: 62 - DNA, 35 bp, Artificial Sequence
  Synthetic oligonucleotide
ttggtgtccctaaaacgagcacgtcttttcaccag

SEQ ID NO: 63 - DNA, 35 bp, Artificial Sequence
  Synthetic oligonucleotide
tagcaatactgcatgcctgcaatcagagcgggagc

SEQ ID NO: 64 - DNA, 28 bp, Artificial Sequence
  Synthetic oligonucleotide
caaaagcggtcagtgtcattgggcctct

SEQ ID NO: 65 - DNA, 49 bp, Artificial Sequence
  Synthetic oligonucleotide
gaacctcgccagttacaaaattaccttttgaaatatatcagaattaaat

SEQ ID NO: 66 - DNA, 35 bp, Artificial Sequence
  Synthetic oligonucleotide
agggaaggcgtaaccaccacaggattttcatcacg

SEQ ID NO: 67 - DNA, 42 bp, Artificial Sequence
  Synthetic oligonucleotide
cccgccggtggcgagaaaggaccattgccttgcctagacttt

SEQ ID NO: 68 - DNA, 42 bp, Artificial Sequence
  Synthetic oligonucleotide
acgtcaagcccttcaccgcctaacgcgcggggagaggcggtt

SEQ ID NO: 69 - DNA, 35 bp, Artificial Sequence
  Synthetic oligonucleotide
tgttttaaatatgcatcaatatatgtgcggatggc

SEQ ID NO: 70 - DNA, 28 bp, Artificial Sequence
  Synthetic oligonucleotide
gtctttatgaacctcaaatatttttaaa

SEQ ID NO: 71 - DNA, 28 bp, Artificial Sequence
  Synthetic oligonucleotide
ccgaccgcgccataagtcctgaacaaga

SEQ ID NO: 72 - DNA, 35 bp, Artificial Sequence
  Synthetic oligonucleotide
ttaagaacgcgagaaaactttaatataagacgacg

SEQ ID NO: 73 - DNA, 35 bp, Artificial Sequence
  Synthetic oligonucleotide
gaacaagagtccacgaagatctacgccaacaaagg

SEQ ID NO: 74 - DNA, 26 bp, Artificial Sequence
  Synthetic oligonucleotide
atcgcccagcagggagttaatgataa

SEQ ID NO: 75 - DNA, 35 bp, Artificial Sequence
  Synthetic oligonucleotide
gcactaaatcggaaagatgggcccagtcagtttga

SEQ ID NO: 76 - DNA, 23 bp, Artificial Sequence
  Synthetic oligonucleotide
acggggtcaggtttatcagcttg

SEQ ID NO: 77 - DNA, 25 bp, Artificial Sequence
  Synthetic oligonucleotide
agtctctgggtaaaatacgtaatgc

SEQ ID NO: 78 - DNA, 49 bp, Artificial Sequence
  Synthetic oligonucleotide
taaagatgtctggaaaagcccaagattgtataagctgttaaatctggtg

SEQ ID NO: 79 - DNA, 35 bp, Artificial Sequence
  Synthetic oligonucleotide
caccgcttcagctcattttttaaccaatagccagc

SEQ ID NO: 80 - DNA, 28 bp, Artificial Sequence
  Synthetic oligonucleotide
ggcgaaccgcttaatgcgccgtaaacag

SEQ ID NO: 81 - DNA, 28 bp, Artificial Sequence
  Synthetic oligonucleotide
aactaaattatttcaacgcaagtgtagg

SEQ ID NO: 82 - DNA, 28 bp, Artificial Sequence
  Synthetic oligonucleotide
ttttgttagcaaatcagatatttacgag

SEQ ID NO: 83 - DNA, 42 bp, Artificial Sequence
  Synthetic oligonucleotide
gagacagccctgtattccatataacagtaatttcaccttaga

SEQ ID NO: 84 - DNA, 28 bp, Artificial Sequence
  Synthetic oligonucleotide
cagtgccaagctttctttgataactcgt

SEQ ID NO: 85 - DNA, 42 bp, Artificial Sequence
  Synthetic oligonucleotide
acaaacatgaaaggtctgacctgaaagctttgacgaaaacgc

SEQ ID NO: 86 - DNA, 21 bp, Artificial Sequence
  Synthetic oligonucleotide
ttcatttcatccaataaatca

SEQ ID NO: 87 - DNA, 49 bp, Artificial Sequence
  Synthetic oligonucleotide
aaaatactgagagccagcagcggagaggtgcaaggctgtttcctgtgtg

SEQ ID NO: 88 - DNA, 42 bp, Artificial Sequence
  Synthetic oligonucleotide
tctgacccaatataatcctgattgtttggattatagatttag

SEQ ID NO: 89 - DNA, 42 bp, Artificial Sequence
  Synthetic oligonucleotide
ggtcgactgagaattgtgatataggtctaattattcatttca

SEQ ID NO: 90 - DNA, 36 bp, Artificial Sequence
  Synthetic oligonucleotide
ttctacaattttatcctggctattttgcacccagtt

SEQ ID NO: 91 - DNA, 21 bp, Artificial Sequence
  Synthetic oligonucleotide
agtttcaatacttttgcggga

SEQ ID NO: 92 - DNA, 32 bp, Artificial Sequence
  Synthetic oligonucleotide
cagaagcagagtacctttaattgctccttttt

SEQ ID NO: 93 - DNA, 42 bp, Artificial Sequence
  Synthetic oligonucleotide
tttaggccaaattaaacatcaaacaggactcaatcgtctgaa

SEQ ID NO: 94 - DNA, 35 bp, Artificial Sequence
  Synthetic oligonucleotide
caaaagaagttttgccagaggttgcttccaggtca

SEQ ID NO: 95 - DNA, 28 bp, Artificial Sequence
  Synthetic oligonucleotide
gctggcgtatccgcttaatgaatcggcc

SEQ ID NO: 96 - DNA, 35 bp, Artificial Sequence
  Synthetic oligonucleotide
cagtttgcacgctggtttgccagtcggggagccgg

SEQ ID NO: 97 - DNA, 28 bp, Artificial Sequence
  Synthetic oligonucleotide
tctatcatgagacgggcaacatgcgtat

SEQ ID NO: 98 - DNA, 31 bp, Artificial Sequence
  Synthetic oligonucleotide
tacaaactccatcgttgacccccagtagcaa

SEQ ID NO: 99 - DNA, 28 bp, Artificial Sequence
  Synthetic oligonucleotide
tcattaccgcgccctcaataaatacaaa

SEQ ID NO: 100 - DNA, 28 bp, Artificial Sequence
  Synthetic oligonucleotide
cgttaaacagtaggtatcccatcctaat

SEQ ID NO: 101 - DNA, 35 bp, Artificial Sequence
  Synthetic oligonucleotide
accagaagcaaaattttcgcaaatggtcattacct

SEQ ID NO: 102 - DNA, 36 bp, Artificial Sequence
  Synthetic oligonucleotide
gaggcgcagacagcaaaatgtatcatcgccaggccg

SEQ ID NO: 103 - DNA, 35 bp, Artificial Sequence
  Synthetic oligonucleotide
gctgattagggcgaaaaaccggcatctggttgggt

SEQ ID NO: 104 - DNA, 35 bp, Artificial Sequence
  Synthetic oligonucleotide
caaaaagactccaatgtaaatgaaacagtacataa

SEQ ID NO: 105 - DNA, 35 bp, Artificial Sequence
  Synthetic oligonucleotide
caagccggcgagaggcttttgattaattcagaccg

SEQ ID NO: 106 - DNA, 42 bp, Artificial Sequence
  Synthetic oligonucleotide
gcttaattctagagtgtaaaaggtcacgcggattctccgtgg

SEQ ID NO: 107 - DNA, 35 bp, Artificial Sequence
  Synthetic oligonucleotide
aaattgtaaaggggagtatcgtcgcgtctggcctt

SEQ ID NO: 108 - DNA, 28 bp, Artificial Sequence
  Synthetic oligonucleotide
taaatttcatgtaacctgtttatcaaca

SEQ ID NO: 109 - DNA, 46 bp, Artificial Sequence
  Synthetic oligonucleotide
ttgctggcaagtgtagcggtccgccagaatcctgagaagtgttttt

SEQ ID NO: 110 - DNA, 35 bp, Artificial Sequence
  Synthetic oligonucleotide
agaaggcaataagaaacgattagagtcaaaacacc

SEQ ID NO: 111 - DNA, 35 bp, Artificial Sequence
  Synthetic oligonucleotide
tgatggcgcattaaggggcgcgagctgataccaag

SEQ ID NO: 112 - DNA, 35 bp, Artificial Sequence
  Synthetic oligonucleotide
aagaacgcatattatttatccaaaatcaaataagg

SEQ ID NO: 113 - DNA, 42 bp, Artificial Sequence
  Synthetic oligonucleotide
aaggccgctatcagattaacaataaaacagaggtgagacagg

SEQ ID NO: 114 - DNA, 28 bp, Artificial Sequence
  Synthetic oligonucleotide
agtagatataaagctaaatcgattcaac

SEQ ID NO: 115 - DNA, 35 bp, Artificial Sequence
  Synthetic oligonucleotide
atctaaaggccaacagagataatggattccgccag

SEQ ID NO: 116 - DNA, 35 bp, Artificial Sequence
  Synthetic oligonucleotide
gtcatagcgattaaccagtttccagctttcatcaa

SEQ ID NO: 117 - DNA, 49 bp, Artificial Sequence
  Synthetic oligonucleotide
agaaaccgtaacataccttgcatgcgcgaactgatcattaaataaccgt

SEQ ID NO: 118 - DNA, 28 bp, Artificial Sequence
  Synthetic oligonucleotide
gagtagagtctgtcagacaggaacggta

SEQ ID NO: 119 - DNA, 36 bp, Artificial Sequence
  Synthetic oligonucleotide
ttagcatgtcaatcatatcggtaatcgtaaaacttt

SEQ ID NO: 120 - DNA, 35 bp, Artificial Sequence
  Synthetic oligonucleotide
atcatattacaggctgtttagctatattagaggcg

SEQ ID NO: 121 - DNA, 39 bp, Artificial Sequence
  Synthetic oligonucleotide
taattacctttaattgtatcgtgccttgagtacaagaaa

SEQ ID NO: 122 - DNA, 35 bp, Artificial Sequence
  Synthetic oligonucleotide
ataaataagtaaaatgtttagactggatagcgttt

SEQ ID NO: 123 - DNA, 36 bp, Artificial Sequence
  Synthetic oligonucleotide
ttgtctttaccctgactaataaatcaaaaatcagtt

SEQ ID NO: 124 - DNA, 42 bp, Artificial Sequence
  Synthetic oligonucleotide
ctacaggtgacggggaaagcctcatggaaagattgaccgtaa

SEQ ID NO: 125 - DNA, 35 bp, Artificial Sequence
  Synthetic oligonucleotide
tttaactcacattaattgcgttgcgctcaagcctg

SEQ ID NO: 126 - DNA, 35 bp, Artificial Sequence
  Synthetic oligonucleotide
acgctgcaaagcgaaaggagcgggcgctagggctt

SEQ ID NO: 127 - DNA, 28 bp, Artificial Sequence
  Synthetic oligonucleotide
tgattcccaaaaacattatgatcaaatc

SEQ ID NO: 128 - DNA, 49 bp, Artificial Sequence
  Synthetic oligonucleotide
aaaaatggcttagatagaaaaagcctgtttagtttaattcgaaccatca

SEQ ID NO: 129 - DNA, 42 bp, Artificial Sequence
  Synthetic oligonucleotide
gccagtataaaagaagaactcaatattaatttacattggcag

SEQ ID NO: 130 - DNA, 35 bp, Artificial Sequence
  Synthetic oligonucleotide
ggtgagagaagcaaattaagaaagtaccgcatgct

SEQ ID NO: 131 - DNA, 42 bp, Artificial Sequence
  Synthetic oligonucleotide
atatgatgttgtaccaattctgcgaacgacaaaatagcgata

SEQ ID NO: 132 - DNA, 35 bp, Artificial Sequence
  Synthetic oligonucleotide
agaggcattcatctgttatatctgattgctttgaa

SEQ ID NO: 133 - DNA, 28 bp, Artificial Sequence
  Synthetic oligonucleotide
ttcaaatgctgatggagaaacaataacg

SEQ ID NO: 134 - DNA, 28 bp, Artificial Sequence
  Synthetic oligonucleotide
agttaatttttcgagttcagctaatgca

SEQ ID NO: 135 - DNA, 28 bp, Artificial Sequence
  Synthetic oligonucleotide
gaaccctaattgaggaaggttaagtatt

SEQ ID NO: 136 - DNA, 42 bp, Artificial Sequence
  Synthetic oligonucleotide
ggccctggaacgtggactccacgacgacgatgtgcgtagcta

SEQ ID NO: 137 - DNA, 35 bp, Artificial Sequence
  Synthetic oligonucleotide
ttttttgttaaaattcgcattaaattttaaatatt

SEQ ID NO: 138 - DNA, 28 bp, Artificial Sequence
  Synthetic oligonucleotide
ggattagaaagcgggttcagaaaacgag

SEQ ID NO: 139 - DNA, 36 bp, Artificial Sequence
  Synthetic oligonucleotide
tttggtaatatccagaacaaactatcggccttgctt

SEQ ID NO: 140 - DNA, 35 bp, Artificial Sequence
  Synthetic oligonucleotide
aaatgaaaaacatcgccattacctgtaggagggga

SEQ ID NO: 141 - DNA, 28 bp, Artificial Sequence
  Synthetic oligonucleotide
aacatacaaacctgtcgtgccagcggtc

SEQ ID NO: 142 - DNA, 42 bp, Artificial Sequence
  Synthetic oligonucleotide
tgctttggggagcccccgatttgggatacgacggcccgaacg

SEQ ID NO: 143 - DNA, 35 bp, Artificial Sequence
  Synthetic oligonucleotide
tttattttaaatgcaatgcctgagtaatggataaa

SEQ ID NO: 144 - DNA, 42 bp, Artificial Sequence
  Synthetic oligonucleotide
tttttgagccacgccgaacgaaccaccaaaataatgcctcag

SEQ ID NO: 145 - DNA, 35 bp, Artificial Sequence
  Synthetic oligonucleotide
acgccaaaatggttttaacctttacaaaatcgcgc

SEQ ID NO: 146 - DNA, 35 bp, Artificial Sequence
  Synthetic oligonucleotide
aaaatagcagacgataaaaacatccttgaaaacat

SEQ ID NO: 147 - DNA, 36 bp, Artificial Sequence
  Synthetic oligonucleotide
ttgaatataatgctgtagttagagcttaattgcttt

SEQ ID NO: 148 - DNA, 44 bp, Artificial Sequence
  Synthetic oligonucleotide
cagtatacatgtagaaaccaaaatagcataacgtccataaaaac

SEQ ID NO: 149 - DNA, 41 bp, Artificial Sequence
  Synthetic oligonucleotide
caagaaacaccaccctccccctttccctcagagcagccacc

SEQ ID NO: 150 - DNA, 40 bp, Artificial Sequence
  Synthetic oligonucleotide
aaaggaatgtctttccagacgttattgcgaataataattt

SEQ ID NO: 151 - DNA, 40 bp, Artificial Sequence
  Synthetic oligonucleotide
cgggagaatgtaacactaatcagcactaaaacactttgag

SEQ ID NO: 152 - DNA, 39 bp, Artificial Sequence
  Synthetic oligonucleotide
gcaacactgcgtaaccattaccaagtacaacgggtcacc

SEQ ID NO: 153 - DNA, 39 bp, Artificial Sequence
  Synthetic oligonucleotide
caaagtcaagcccaataagtttaaagaggcaaattcatg

SEQ ID NO: 154 - DNA, 41 bp, Artificial Sequence
  Synthetic oligonucleotide
tatcttacccgtactcaatctttccaccaccggagccacca

SEQ ID NO: 155 - DNA, 34 bp, Artificial Sequence
  Synthetic oligonucleotide
attgagttagaaccgccggcatccctcagacact

SEQ ID NO: 156 - DNA, 41 bp, Artificial Sequence
  Synthetic oligonucleotide
aacaaataaatcctccggggttttccaccctcaagcccaat

SEQ ID NO: 157 - DNA, 49 bp, Artificial Sequence
  Synthetic oligonucleotide
attaaagccagaatggaaagcgctcctcaagaagagccacagagataac

SEQ ID NO: 158 - DNA, 36 bp, Artificial Sequence
  Synthetic oligonucleotide
taccacattcaactaataattttctcggaacattgt

SEQ ID NO: 159 - DNA, 44 bp, Artificial Sequence; identical to SEQ ID NO: 148
  Synthetic oligonucleotide

SEQ ID NO: 160 - DNA, 39 bp, Artificial Sequence
  Synthetic oligonucleotide
gacgattggccttgataagtgcctagtaccgatgaaata

SEQ ID NO: 161 - DNA, 30 bp, Artificial Sequence
  Synthetic oligonucleotide
aatttaccgttccagcatgaaaggatagca

SEQ ID NO: 162 - DNA, 38 bp, Artificial Sequence
  Synthetic oligonucleotide
attttgctaaacaactttataggtgtatcacgaagccc

SEQ ID NO: 163 - DNA, 50 bp, Artificial Sequence
  Synthetic oligonucleotide
tttttaaatcagttgagatttaggaattacaggtagaaagattcgaaaag

SEQ ID NO: 164 - DNA, 50 bp, Artificial Sequence
  Synthetic oligonucleotide
gtcgaagaggcttcgcataaccgatatattagcattgacaggaggttgag

SEQ ID NO: 165 - DNA, 36 bp, Artificial Sequence
  Synthetic oligonucleotide
gagccgccgcccggtcgctatccgcgaccaccggaa

SEQ ID NO: 166 - DNA, 20 bp, Artificial Sequence
  Synthetic oligonucleotide
cgctgttcctcacgataatt

SEQ ID NO: 167 - DNA, 20 bp, Artificial Sequence
  Synthetic oligonucleotide
tttagcttccataccacctg

SEQ ID NO: 168 - DNA, 49 bp, Artificial Sequence
  Synthetic oligonucleotide
atcggaacgagggcgatttcaccagtgaattcaggtggtatggaagcta

SEQ ID NO: 169 - DNA, 56 bp, Artificial Sequence
  Synthetic oligonucleotide
cttaaacctcagcagcgaaaaaacaattagcccgacttcaggtggtatggaagcta

SEQ ID NO: 170 - DNA, 50 bp, Artificial Sequence
  Synthetic oligonucleotide
accgccaccctcagcgccatttcgggtttattcaggtggtatggaagcta

SEQ ID NO: 171 - DNA, 60 bp, Artificial Sequence
  Synthetic oligonucleotide
aagttttacggctacagaggctcatctatagcaggaaattttcaggtggtatggaagcta

SEQ ID NO: 172 - DNA, 58 bp, Artificial Sequence
  Synthetic oligonucleotide
tattcacaaccctcagagccaccgccattagcaatagattcaggtggtatggaagcta

SEQ ID NO: 173 - DNA, 45 bp, Artificial Sequence
  Synthetic oligonucleotide
caccctcagactgtagcgcgacaaattcaggtggtatggaagcta

SEQ ID NO: 174 - DNA, 60 bp, Artificial Sequence
  Synthetic oligonucleotide
tgatacaggactaaagactttagaatatagcgacgaaggtttcaggtggtatggaagcta

SEQ ID NO: 175 - DNA, 60 bp, Artificial Sequence
  Synthetic oligonucleotide
taagcgtcaggaagtttccataaaacggcctttacaaccgttcaggtggtatggaagcta

SEQ ID NO: 176 - DNA, 58 bp, Artificial Sequence
  Synthetic oligonucleotide
ttgcgcccttttgcgggatcagatttcaccaggggaatttcaggtggtatggaagcta

SEQ ID NO: 177 - DNA, 59 bp, Artificial Sequence
  Synthetic oligonucleotide
ggaagaaaaatctaccgcatagtagagccggtcaatcatttcaggtggtatggaagcta

SEQ ID NO: 178 - DNA, 58 bp, Artificial Sequence
  Synthetic oligonucleotide
gcaggtcagaaccaccaccaccagagtcataatttattttcaggtggtatggaagcta

SEQ ID NO: 179 - DNA, 63 bp, Artificial Sequence
  Synthetic oligonucleotide
agacgcctttacagacttatgcgattttaacaagaacttatcattcaggtggtatggaagcta

SEQ ID NO: 180 - DNA, 47 bp, Artificial Sequence
  Synthetic oligonucleotide
aacgaactaacggaacaacggtaagggttcaggtggtatggaagcta

SEQ ID NO: 181 - DNA, 48 bp, Artificial Sequence
  Synthetic oligonucleotide
gcaataataacggaatacgtagccagcgttcaggtggtatggaagcta

SEQ ID NO: 182 - DNA, 48 bp, Artificial Sequence
  Synthetic oligonucleotide
tcattataccagtcatcatcaattgagcttcaggtggtatggaagcta

SEQ ID NO: 183 - DNA, 46 bp, Artificial Sequence
  Synthetic oligonucleotide
ttgggcttgagatggagctgcaaatattcaggtggtatggaagcta

SEQ ID NO: 184 - DNA, 46 bp, Artificial Sequence
  Synthetic oligonucleotide
taagcagatagccgaagaaacttgtcttcaggtggtatggaagcta

SEQ ID NO: 185 - DNA, 48 bp, Artificial Sequence
  Synthetic oligonucleotide
agaactggcatgattattacgcagggcgttcaggtggtatggaagcta

SEQ ID NO: 186 - DNA, 47 bp, Artificial Sequence
  Synthetic oligonucleotide
taccagaaggaaaccgaaaggtaaattttcaggtggtatggaagcta

SEQ ID NO: 187 - DNA, 46 bp, Artificial Sequence
  Synthetic oligonucleotide
caactttaatcattgacccaaattcattcaggtggtatggaagcta

SEQ ID NO: 188 - DNA, 55 bp, Artificial Sequence
  Synthetic oligonucleotide
gagggtaagaaacaccagaacgaaaggctattgagttcaggtggtatggaagcta

SEQ ID NO: 189 - DNA, 58 bp, Artificial Sequence
  Synthetic oligonucleotide
gagtgtactggtaatgtataaactcaccagagggaagcttttatcgtgaggaacagcg

SEQ ID NO: 190 - DNA, 58 bp, Artificial Sequence
  Synthetic oligonucleotide
atacatggcttttgatatttcggatgtacctaactgaattttatcgtgaggaacagcg

SEQ ID NO: 191 - DNA, 60 bp, Artificial Sequence
  Synthetic oligonucleotide
gacaatgacaacaaccctaaaggaagtaaatggcagatacttttatcgtgaggaacagcg

SEQ ID NO: 192 - DNA, 60 bp, Artificial Sequence
  Synthetic oligonucleotide
agcttgataccgatagtttcacgtgttttgtctacgaggcttttatcgtgaggaacagcg

SEQ ID NO: 193 - DNA, 57 bp, Artificial Sequence
  Synthetic oligonucleotide
ccgtcaaaggccacagccctcatagttaatcataaccttttatcgtgaggaacagcg

SEQ ID NO: 194 - DNA, 69 bp, Artificial Sequence
  Synthetic oligonucleotide
attaaagccagaatggaaagcgctcctcaagaagagccacagagataacttttatcgtgaggaacagcg

SEQ ID NO: 195 - DNA, 61 bp, Artificial Sequence
  Synthetic oligonucleotide
aacaaataaatcctccggggttttccaccctcaagcccaatttttatcgtgaggaacagcg

SEQ ID NO: 196 - DNA, 59 bp, Artificial Sequence
  Synthetic oligonucleotide
gacgattggccttgataagtgcctagtaccgatgaaatattttatcgtgaggaacagcg

SEQ ID NO: 197 - DNA, 7249 bp, Artificial Sequence
  Synthetic oligonucleotide
aatgctactactattagtagaattgatgccaccttttcagctcgcgccccaaatgaaaatatagctaaacaggttattgaccatttgcgaaatgtatctaatggtcaaactaaatctactcgttcgcagaattgggaatcaactgttatatggaatgaaacttccagacaccgtactttagttgcatatttaaaacatgttgagctacagcattatattcagcaattaagctctaagccatccgcaaaaatgacctcttatcaaaaggagcaattaaaggtactctctaatcctgacctgttggagtttgcttccggtctggttcgctttgaagctcgaattaaaacgcgatatttgaagtctttcgggcttcctcttaatctttttgatgcaatccgctttgcttctgactataatagtcagggtaaagacctgatttttgatttatggtcattctcgttttctgaactgtttaaagcatttgagggggattcaatgaatatttatgacgattccgcagtattggacgctatccagtctaaacattttactattaccccctctggcaaaacttcttttgcaaaagcctctcgctattttggtttttatcgtcgtctggtaaacgagggttatgatagtgttgctcttactatgcctcgtaattccttttggcgttatgtatctgcattagttgaatgtggtattcctaaatctcaactgatgaatctttctacctgtaataatgttgttccgttagttcgttttattaacgtagatttttcttcccaacgtcctgactggtataatgagccagttcttaaaatcgcataaggtaattcacaatgattaaagttgaaattaaaccatctcaagcccaatttactactcgttctggtgtttctcgtcagggcaagccttattcactgaatgagcagctttgttacgttgatttgggtaatgaatatccggttcttgtcaagattactcttgatgaaggtcagccagcctatgcgcctggtctgtacaccgttcatctgtcctctttcaaagttggtcagttcggttcccttatgattgaccgtctgcgcctcgttccggctaagtaacatggagcaggtcgcggatttcgacacaatttatcaggcgatgatacaaatctccgttgtactttgtttcgcgcttggtataatcgctgggggtcaaagatgagtgttttagtgtattcttttgcctctttcgttttaggttggtgccttcgtagtggcattacgtattttacccgtttaatggaaacttcctcatgaaaaagtctttagtcctcaaagcctctgtagccgttgctaccctcgttccgatgctgtctttcgctgctgagggtgacgatcccgcaaaagcggcctttaactccctgcaagcctcagcgaccgaatatatcggttatgcgtgggcgatggttgttgtcattgtcggcgcaactatcggtatcaagctgtttaagaaattcacctcgaaagcaagctgataaaccgatacaattaaaggctccttttggagccttttttttggagattttcaacgtgaaaaaattattattcgcaattcctttagttgttcctttctattctcactccgctgaaactgttgaaagttgtttagcaaaatcccatacagaaaattcatttactaacgtctggaaagacgacaaaactttagatcgttacgctaactatgagggctgtctgtggaatgctacaggcgttgtagtttgtactggtgacgaaactcagtgttacggtacatgggttcctattgggcttgctatccctgaaaatgagggtggtggctctgagggtggcggttctgagggtggcggttctgagggtggcggtactaaacctcctgagtacggtgatacacctattccgggctatacttatatcaaccctctcgacggcacttatccgcctggtactgagcaaaaccccgctaatcctaatccttctcttgaggagtctcagcctcttaatactttcatgtttcagaataataggttccgaaataggcagggggcattaactgtttatacgggcactgttactcaaggcactgaccccgttaaaacttattaccagtacactcctgtatcatcaaaagccatgtatgacgcttactggaacggtaaattcagagactgcgctttccattctggctttaatgaggatttatttgtttgtgaatatcaaggccaatcgtctgacctgcctcaacctcctgtcaatgctggcggcggctctggtggtggttctggtggcggctctgagggtggtggctctgagggtggcggttctgagggtggcggctctgagggaggcggttccggtggtggctctggttccggtgattttgattatgaaaagatggcaaacgctaataagggggctatgaccgaaaatgccgatgaaaacgcgctacagtctgacgctaaaggcaaacttgattctgtcgctactgattacggtgctgctatcgatggtttcattggtgacgtttccggccttgctaatggtaatggtgctactggtgattttgctggctctaattcccaaatggctcaagtcggtgacggtgataattcacctttaatgaataatttccgtcaatatttaccttccctccctcaatcggttgaatgtcgcccttttgtctttggcgctggtaaaccatatgaattttctattgattgtgacaaaataaacttattccgtggtgtctttgcgtttcttttatatgttgccacctttatgtatgtattttctacgtttgctaacatactgcgtaataaggagtcttaatcatgccagttcttttgggtattccgttattattgcgtttcctcggtttccttctggtaactttgttcggctatctgcttacttttcttaaaaagggcttcggtaagatagctattgctatttcattgtttcttgctcttattattgggcttaactcaattcttgtgggttatctctctgatattagcgctcaattaccctctgactttgttcagggtgttcagttaattctcccgtctaatgcgcttccctgtttttatgttattctctctgtaaaggctgctattttcatttttgacgttaaacaaaaaatcgtttcttatttggattgggataaataatatggctgtttattttgtaactggcaaattaggctctggaaagacgctcgttagcgttggtaagattcaggataaaattgtagctgggtgcaaaatagcaactaatcttgatttaaggcttcaaaacctcccgcaagtcgggaggttcgctaaaacgcctcgcgttcttagaataccggataagccttctatatctgatttgcttgctattgggcgcggtaatgattcctacgatgaaaataaaaacggcttgcttgttctcgatgagtgcggtacttggtttaatacccgttcttggaatgataaggaaagacagccgattattgattggtttctacatgctcgtaaattaggatgggatattatttttcttgttcaggacttatctattgttgataaacaggcgcgttctgcattagctgaacatgttgtttattgtcgtcgtctggacagaattactttaccttttgtcggtactttatattctcttattactggctcgaaaatgcctctgcctaaattacatgttggcgttgttaaatatggcgattctcaattaagccctactgttgagcgttggctttatactggtaagaatttgtataacgcatatgatactaaacaggctttttctagtaattatgattccggtgtttattcttatttaacgccttatttatcacacggtcggtatttcaaaccattaaatttaggtcagaagatgaaattaactaaaatatatttgaaaaagttttctcgcgttctttgtcttgcgattggatttgcatcagcatttacatatagttatataacccaacctaagccggaggttaaaaaggtagtctctcagacctatgattttgataaattcactattgactcttctcagcgtcttaatctaagctatcgctatgttttcaaggattctaagggaaaattaattaatagcgacgatttacagaagcaaggttattcactcacatatattgatttatgtactgtttccattaaaaaaggtaattcaaatgaaattgttaaatgtaattaattttgttttcttgatgtttgtttcatcatcttcttttgctcaggtaattgaaatgaataattcgcctctgcgcgattttgtaacttggtattcaaagcaatcaggcgaatccgttattgtttctcccgatgtaaaaggtactgttactgtatattcatctgacgttaaacctgaaaatctacgcaatttctttatttctgttttacgtgcaaataattttgatatggtaggttctaacccttccattattcagaagtataatccaaacaatcaggattatattgatgaattgccatcatctgataatcaggaatatgatgataattccgctccttctggtggtttctttgttccgcaaaatgataatgttactcaaacttttaaaattaataacgttcgggcaaaggatttaatacgagttgtcgaattgtttgtaaagtctaatacttctaaatcctcaaatgtattatctattgacggctctaatctattagttgttagtgctcctaaagatattttagataaccttcctcaattcctttcaactgttgatttgccaactgaccagatattgattgagggtttgatatttgaggttcagcaaggtgatgctttagatttttcatttgctgctggctctcagcgtggcactgttgcaggcggtgttaatactgaccgcctcacctctgttttatcttctgctggtggttcgttcggtatttttaatggcgatgttttagggctatcagttcgcgcattaaagactaatagccattcaaaaatattgtctgtgccacgtattcttacgctttcaggtcagaagggttctatctctgttggccagaatgtcccttttattactggtcgtgtgactggtgaatctgccaatgtaaataatccatttcagacgattgagcgtcaaaatgtaggtatttccatgagcgtttttcctgttgcaatggctggcggtaatattgttctggatattaccagcaaggccgatagtttgagttcttctactcaggcaagtgatgttattactaatcaaagaagtattgctacaacggttaatttgcgtgatggacagactcttttactcggtggcctcactgattataaaaacacttctcaggattctggcgtaccgttcctgtctaaaatccctttaatcggcctcctgtttagctcccgctctgattctaacgaggaaagcacgttatacgtgctcgtcaaagcaaccatagtacgcgccctgtagcggcgcattaagcgcggcgggtgtggtggttacgcgcagcgtgaccgctacacttgccagcgccctagcgcccgctcctttcgctttcttcccttcctttctcgccacgttcgccggctttccccgtcaagctctaaatcgggggctccctttagggttccgatttagtgctttacggcacctcgaccccaaaaaacttgatttgggtgatggttcacgtagtgggccatcgccctgatagacggtttttcgccctttgacgttggagtccacgttctttaatagtggactcttgttccaaactggaacaacactcaaccctatctcgggctattcttttgatttataagggattttgccgatttcggaaccaccatcaaacaggattttcgcctgctggggcaaaccagcgtggaccgcttgctgcaactctctcagggccaggcggtgaagggcaatcagctgttgcccgtctcactggtgaaaagaaaaaccaccctggcgcccaatacgcaaaccgcctctccccgcgcgttggccgattcattaatgcagctggcacgacaggtttcccgactggaaagcgggcagtgagcgcaacgcaattaatgtgagttagctcactcattaggcaccccaggctttacactttatgcttccggctcgtatgttgtgtggaattgtgagcggataacaatttcacacaggaaacagctatgaccatgattacgaattcgagctcggtacccggggatcctctagagtcgacctgcaggcatgcaagcttggcactggccgtcgttttacaacgtcgtgactgggaaaaccctggcgttacccaacttaatcgccttgcagcacatccccctttcgccagctggcgtaatagcgaagaggcccgcaccgatcgcccttcccaacagttgcgcagcctgaatggcgaatggcgctttgcctggtttccggcaccagaagcggtgccggaaagctggctggagtgcgatcttcctgaggccgatactgtcgtcgtcccctcaaactggcagatgcacggttacgatgcgcccatctacaccaacgtgacctatcccattacggtcaatccgccgtttgttcccacggagaatccgacgggttgttactcgctcacatttaatgttgatgaaagctggctacaggaaggccagacgcgaattatttttgatggcgttcctattggttaaaaaatgagctgatttaacaaaaatttaatgcgaattttaacaaaatattaacgtttacaatttaaatatttgcttatacaatcttcctgtttttggggcttttctgattatcaaccggggtacatatgattgacatgctagttttacgattaccgttcatcgattctcttgtttgctccagactctcaggcaatgacctgatagcctttgtagatctctcaaaaatagctaccctctccggcattaatttatcagctagaacggttgaatatcatattgatggtgatttgactgtctccggcctttctcacccttttgaatctttacctacacattactcaggcattgcatttaaaatatatgagggttctaaaaatttttatccttgcgttgaaataaaggcttctcccgcaaaagtattacagggtcataatgtttttggtacaaccgatttagctttatgctctgaggctttattgcttaattttgctaattctttgccttgcctgtatgatttattggatgtt